European Patent Application EP 4 365 199 A1, published May 8, 2024. Title: CD16 ANTIBODY AND USE THEREOF. Applicant: JIANGSU SIMCERE PHARMACEUTICAL CO., LTD. Application EP22831997.6. The sequence listing filed with the application follows.

SEQUENCE LISTING (113 sequences)

SEQ ID NO: 1 - protein, 254 aa, Homo sapiens
MWQLLLPTALLLLVSAGMRTEDLPKAVVFLEPQWYRVLEKDSVTLKCQGAYSPEDNSTQWFHNESLISSQASSYFIDAATVDDSGEYRCQTNLSTLSDPVQLEVHIGWLLLQAPRWVFKEEDPIHLRCHSWKNTALHKVTYLQNGKGRKYFHHNSDFYIPKATLKDSGSYFCRGLFGSKNVSSETVNITITQGLAVSTISSFFPPGYQVSFCLVMVLLFAVDTGLYFSVKTNIRSSTRDWKDHKFKWRKDPQDK

SEQ ID NO: 2 - protein, 254 aa, Homo sapiens
MWQLLLPTALLLLVSAGMRTEDLPKAVVFLEPQWYRVLEKDSVTLKCQGAYSPEDNSTQWFHNESLISSQASSYFIDAATVDDSGEYRCQTNLSTLSDPVQLEVHIGWLLLQAPRWVFKEEDPIHLRCHSWKNTALHKVTYLQNGKGRKYFHHNSDFYIPKATLKDSGSYFCRGLVGSKNVSSETVNITITQGLAVSTISSFFPPGYQVSFCLVMVLLFAVDTGLYFSVKTNIRSSTRDWKDHKFKWRKDPQDK

SEQ ID NO: 3 - protein, 233 aa, Homo sapiens
MWQLLLPTALLLLVSAGMRTEDLPKAVVFLEPQWYRVLEKDSVTLKCQGAYSPEDNSTQWFHNENLISSQASSYFIDAATVDDSGEYRCQTNLSTLSDPVQLEVHVGWLLLQAPRWVFKEEDPIHLRCHSWKNTALHKVTYLQNGKDRKYFHHNSDFHIPKATLKDSGSYFCRGLVGSKNVSSETVNITITQGLAVSTISSFSPPGYQVSFCLVMVLLFAVDTGLYFSVKTNI

SEQ ID NO: 4 - protein, 233 aa, Homo sapiens
MWQLLLPTALLLLVSAGMRTEDLPKAVVFLEPQWYSVLEKDSVTLKCQGAYSPEDNSTQWFHNESLISSQASSYFIDAATVNDSGEYRCQTNLSTLSDPVQLEVHIGWLLLQAPRWVFKEEDPIHLRCHSWKNTALHKVTYLQNGKDRKYFHHNSDFHIPKATLKDSGSYFCRGLVGSKNVSSETVNITITQGLAVSTISSFSPPGYQVSFCLVMVLLFAVDTGLYFSVKTNI

SEQ ID NO: 5 - protein, 233 aa, Homo sapiens
MWQLLLPTALLLLVSAGMRTEDLPKAVVFLEPQWYSVLEKDSVTLKCQGAYSPEDNSTQWFHNESLISSQASSYFIDDATVNDSGEYRCQTNLSTLSDPVQLEVHIGWLLLQAPRWVFKEEDPIHLRCHSWKNTALHKVTYLQNGKDRKYFHHNSDFHIPKATLKDSGSYFCRGLVGSKNVSSETVNITITQGLAVSTISSFSPPGYQVSFCLVMVLLFAVDTGLYFSVKTNI

SEQ ID NO: 6 - protein, 254 aa, Macaca fascicularis
MWQLLLPTALLLLVSAGMRAEDLPRAVVFLEPQWYRVLEKDRVTLKCQGAYSPEDNSTRWFHNESLISSQTSSYFIAAARVNNSGEYRCQTSLSTLSDPVQLEVHIGWLLLQAPRWVFKEEESIHLRCHSWKNTLLHKVTYLQNGKGRKYFHQNSDFYIPKATLKDSGSYFCRGLIGSKNVSSETVNITITQDLAVSSISSFFPPGYQVSFCLVMVLLFAVDTGLYFSMKKSIPSSTRDWEDHKFKWSKDPQDK

SEQ ID NO: 7 - protein, 424 aa, Artificial Sequence
  Synthetic polypeptide
GMRTEDLPKAVVFLEPQWYRVLEKDSVTLKCQGAYSPEDNSTQWFHNESLISSQASSYFIDAATVDDSGEYRCQTNLSTLSDPVQLEVHIGWLLLQAPRWVFKEEDPIHLRCHSWKNTALHKVTYLQNGKGRKYFHHNSDFYIPKATLKDSGSYFCRGLFGSKNVSSETVNITITQGLAVSTISSFFPPGYQEPKSADKTHTCPPCPAPELLGGPSVFLFPPKPKDTLMISRTPEVTCVVVDVSHEDPEVKFNWYVDGVEVHNAKTKPREEQYASTYRVVSVLTVLHQDWLNGKEYKCKVSNKALPAPIEKTISKAKGQPREPQVYTLPPSREEMTKNQVSLTCLVKGFYPSDIAVEWESNGQPENNYKTTPPVLDSDGSFFLYSKLTVDKSRWQQGNVFSCSVMHEALHNHYTQKSLSLSPGK

SEQ ID NO: 8 - protein, 424 aa, Artificial Sequence
  Synthetic polypeptide
GMRTEDLPKAVVFLEPQWYRVLEKDSVTLKCQGAYSPEDNSTQWFHNESLISSQASSYFIDAATVDDSGEYRCQTNLSTLSDPVQLEVHIGWLLLQAPRWVFKEEDPIHLRCHSWKNTALHKVTYLQNGKGRKYFHHNSDFYIPKATLKDSGSYFCRGLVGSKNVSSETVNITITQGLAVSTISSFFPPGYQEPKSADKTHTCPPCPAPELLGGPSVFLFPPKPKDTLMISRTPEVTCVVVDVSHEDPEVKFNWYVDGVEVHNAKTKPREEQYASTYRVVSVLTVLHQDWLNGKEYKCKVSNKALPAPIEKTISKAKGQPREPQVYTLPPSREEMTKNQVSLTCLVKGFYPSDIAVEWESNGQPENNYKTTPPVLDSDGSFFLYSKLTVDKSRWQQGNVFSCSVMHEALHNHYTQKSLSLSPGK

SEQ ID NO: 9 - protein, 225 aa, Artificial Sequence
  Synthetic polypeptide
GMRTEDLPKAVVFLEPQWYRVLEKDSVTLKCQGAYSPEDNSTQWFHNESLISSQASSYFIDAATVDDSGEYRCQTNLSTLSDPVQLEVHIGWLLLQAPRWVFKEEDPIHLRCHSWKNTALHKVTYLQNGKGRKYFHHNSDFYIPKATLKDSGSYFCRGLFGSKNVSSETVNITITQGLAVSTISSFFPPGYQGLNDIFEAQKIEWHEGGGSGGGSHHHHHHHHHH

SEQ ID NO: 10 - protein, 225 aa, Artificial Sequence
  Synthetic polypeptide
GMRTEDLPKAVVFLEPQWYRVLEKDSVTLKCQGAYSPEDNSTQWFHNESLISSQASSYFIDAATVDDSGEYRCQTNLSTLSDPVQLEVHIGWLLLQAPRWVFKEEDPIHLRCHSWKNTALHKVTYLQNGKGRKYFHHNSDFYIPKATLKDSGSYFCRGLVGSKNVSSETVNITITQGLAVSTISSFFPPGYQGLNDIFEAQKIEWHEGGGSGGGSHHHHHHHHHH

SEQ ID NO: 11 - protein, 217 aa, Artificial Sequence
  Synthetic polypeptide
GMRTEDLPKAVVFLEPQWYRVLEKDSVTLKCQGAYSPEDNSTQWFHNENLISSQASSYFIDAATVDDSGEYRCQTNLSTLSDPVQLEVHVGWLLLQAPRWVFKEEDPIHLRCHSWKNTALHKVTYLQNGKDRKYFHHNSDFHIPKATLKDSGSYFCRGLVGSKNVSSETVNITITQGLAVSTISGGGSGGGSHHHHHHHHHHGLNDIFEAQKIEWHE

SEQ ID NO: 12 - protein, 217 aa, Artificial Sequence
  Synthetic polypeptide
GMRTEDLPKAVVFLEPQWYSVLEKDSVTLKCQGAYSPEDNSTQWFHNESLISSQASSYFIDAATVNDSGEYRCQTNLSTLSDPVQLEVHIGWLLLQAPRWVFKEEDPIHLRCHSWKNTALHKVTYLQNGKDRKYFHHNSDFHIPKATLKDSGSYFCRGLVGSKNVSSETVNITITQGLAVSTISGGGSGGGSHHHHHHHHHHGLNDIFEAQKIEWHE

SEQ ID NO: 13 - protein, 217 aa, Artificial Sequence
  Synthetic polypeptide
GMRTEDLPKAVVFLEPQWYSVLEKDSVTLKCQGAYSPEDNSTQWFHNESLISSQASSYFIDDATVNDSGEYRCQTNLSTLSDPVQLEVHIGWLLLQAPRWVFKEEDPIHLRCHSWKNTALHKVTYLQNGKDRKYFHHNSDFHIPKATLKDSGSYFCRGLVGSKNVSSETVNITITQGLAVSTISGGGSGGGSHHHHHHHHHHGLNDIFEAQKIEWHE

SEQ ID NO: 14 - protein, 225 aa, Artificial Sequence
  Synthetic polypeptide
GMRAEDLPRAVVFLEPQWYRVLEKDRVTLKCQGAYSPEDNSTRWFHNESLISSQTSSYFIAAARVNNSGEYRCQTSLSTLSDPVQLEVHIGWLLLQAPRWVFKEEESIHLRCHSWKNTLLHKVTYLQNGKGRKYFHQNSDFYIPKATLKDSGSYFCRGLIGSKNVSSETVNITITQDLAVSSISSFFPPGYQGLNDIFEAQKIEWHEGGGSGGGSHHHHHHHHHH

SEQ ID NO: 15 - protein, 111 aa, Artificial Sequence
  Synthetic polypeptide
DTVLTQSPASLAVSLGQRATISCKASQSVDFDGDSFMNWYQQKPGQPPKLLIYTTSNLESGIPARFSASGSGTDFTLNIHPVEEEDTATYYCQQSNEDPYTFGGGTKLEIK

SEQ ID NO: 16 - protein, 118 aa, Artificial Sequence
  Synthetic polypeptide
QVTLKESGPGILQPSQTLSLTCSFSGFSLRTSGMGVGWIRQPSGKGLEWLAHIWWDDDKRYNPALKSRLTISKDTSSNQVFLKIASVDTADTATYYCAQINPAWFAYWGQGTLVTVSA

SEQ ID NO: 17 - protein, 476 aa, Artificial Sequence
  Synthetic polypeptide
DTVLTQSPASLAVSLGQRATISCKASQSVDFDGDSFMNWYQQKPGQPPKLLIYTTSNLESGIPARFSASGSGTDFTLNIHPVEEEDTATYYCQQSNEDPYTFGGGTKLEIKGGGGSGGGGSGGGGSQVTLKESGPGILQPSQTLSLTCSFSGFSLRTSGMGVGWIRQPSGKGLEWLAHIWWDDDKRYNPALKSRLTISKDTSSNQVFLKIASVDTADTATYYCAQINPAWFAYWGQGTLVTVSAEPKSSDKTHTCPPCPAPEEFGGPSVFLFPPKPKDTLMISRTPEVTCVVVAVSHEDPEVKFNWYVDGVEVHNAKTKPREEQYNSTYRVVSVLTVLHQDWLNGKEYKCKVSNKALPAPIEKTISKAKGQPREPQVYTLPPSREEMTKNQVSLTCLVKGFYPSDIAVEWESNGQPENNYKTTPPVLDSDGSFFLYSKLTVDKSRWQQGNVFSCSVMHEALHNHYTQKSLSLSPGK

SEQ ID NO: 18 - protein, 120 aa, Artificial Sequence
  Synthetic polypeptide
QVQLVQSGAEVKKPGESLKVSCKASGYTFTSYYMHWVRQAPGQGLEWMGAIEPMYGSTSYAQKFQGRVTMTRDTSTSTVYMELSSLRSEDTAVYYCARGSAYYYDFADYWGQGTLVTVSS

SEQ ID NO: 19 - protein, 106 aa, Artificial Sequence
  Synthetic polypeptide
SYVLTQPSSVSVAPGQTATISCGGHNIGSKNVHWYQQRPGQSPVLVIYQDNKRPSGIPERFSGSNSGNTATLTISGTQAMDEADYYCQVWDNYSVLFGGGTKLTVL

SEQ ID NO: 20 - protein, 473 aa, Artificial Sequence
  Synthetic polypeptide
SYVLTQPSSVSVAPGQTATISCGGHNIGSKNVHWYQQRPGQSPVLVIYQDNKRPSGIPERFSGSNSGNTATLTISGTQAMDEADYYCQVWDNYSVLFGGGTKLTVLGGGGSGGGGSGGGGSQVQLVQSGAEVKKPGESLKVSCKASGYTFTSYYMHWVRQAPGQGLEWMGAIEPMYGSTSYAQKFQGRVTMTRDTSTSTVYMELSSLRSEDTAVYYCARGSAYYYDFADYWGQGTLVTVSSEPKSSDKTHTCPPCPAPEEFGGPSVFLFPPKPKDTLMISRTPEVTCVVVAVSHEDPEVKFNWYVDGVEVHNAKTKPREEQYNSTYRVVSVLTVLHQDWLNGKEYKCKVSNKALPAPIEKTISKAKGQPREPQVYTLPPSREEMTKNQVSLTCLVKGFYPSDIAVEWESNGQPENNYKTTPPVLDSDGSFFLYSKLTVDKSRWQQGNVFSCSVMHEALHNHYTQKSLSLSPGK

SEQ ID NO: 21 - protein, 112 aa, Artificial Sequence
  Synthetic polypeptide
QVQLVESGGGLVQAGGSLRLSCVASRSTLTTYAVRWYRQAPGKQREWVAFISVDGNTNYPDSVKGRFIVSRDNAKNTVYLQMNSLKPEDTADYICRAGGQYWGQGTQVTVSS

SEQ ID NO: 22 - protein, 122 aa, Artificial Sequence
  Synthetic polypeptide
EVQLVESGGGLVQAGGSLRLSCATSGITFSSYAMGWYRQAPGKQRELVAGINRFGLTNYADSVKGRFTISRDNAKNTVYLQMTSLKSEDTAVYYCNTGGVYSHPNYYTGIYWGQGTQVTVSS

SEQ ID NO: 23 - protein, 112 aa, Artificial Sequence
  Synthetic polypeptide
QVQLVESGGGLVQAGGSLRLSCVGSSSTLTTYAVRWYRQAPGKQREWVAFISVDGNTNYPDSVKGRFIVSRDNAKNTVYLQMNNLKPEDTADYICRAGGQYWGQGTQVTVSS

SEQ ID NO: 24 - protein, 112 aa, Artificial Sequence
  Synthetic polypeptide
QVQLVESGGGLVQAGGSLRLSCVASSSTVTTYAVRWYRQAPGKQREWVAFISVDGNTNYPDSVKGRFIVSRDNAKNTVYLQMNSLKPEDTADYICRAGGQYWGQGTQVTVSS

SEQ ID NO: 25 - protein, 112 aa, Artificial Sequence
  Synthetic polypeptide
EVQLVESGGGLVQAGGSLRLSCVASGSTWTTYAVRWYRQAPGKQREWVAFISVDGSTNYPDSVKGRFIVSRDNAKNTVYLQMNSLKPEDTADYICRVGGQYWGQGTQVTVSS

SEQ ID NO: 26 - protein, 112 aa, Artificial Sequence
  Synthetic polypeptide
EVQLVESGGGLVQAGGSLRLSCVASRSTLTTYAVRWYRQAPGKQREWVAFISVDGKTNYPDSVKGRFIVSRDNAKNTVYLQMNSLKPEDTADYICRAGGQYWGQGTQVTVSS

SEQ ID NO: 27 - protein, 112 aa, Artificial Sequence
  Synthetic polypeptide
EVQVVESGGGLVQAGGSLRLSCVASRSTLSTYAVRWYRQAPGNQREWVAFISVDGNTNYPDSVKGRFIVSRDNAKNTVYLQMNSLKPEDTADYICRAGGQYWGQGTQVTVSS

SEQ ID NO: 28 - protein, 112 aa, Artificial Sequence
  Synthetic polypeptide
EVQVVESGGGLVQAGGSLRLSCVASTSTLTTYAVRWYRQAPGKQREWVAFISVDGNTNYPDSVKGRFIVSRDNAKNTVYLQMNSLKPEDTADYICRAGGQYWGQGTQVTVSS

SEQ ID NO: 29 - protein, 112 aa, Artificial Sequence
  Synthetic polypeptide
QVQLVESGGGLVQAGGSLRLSCVGSSSTLTTYAVRWYRQAPGKQREWVAFISVDGSTNYPDSVKGRFIVSRDNAKNTVYLQMNSLKPEDTADYICRAGGQYWGQGTQVTVSS

SEQ ID NO: 30 - protein, 122 aa, Artificial Sequence
  Synthetic polypeptide
EVQVVESGGGLAQAGGSLRLSCAVSGITFSSYAMGWYRQDPGKQRELVAAINRFGLTNYADSVKGRFTISRDNAKNTVYLQMTSLKPEDTAVYYCNTGGVYSHPNYYTGTYWGQGTQVTVSS

SEQ ID NO: 31 - protein, 122 aa, Artificial Sequence
  Synthetic polypeptide
QVQLVESGGGLVQAGGSLRLSCAASGITFSSYAMGWYRQAPGKQRELVAAINRFGLTNYADFVKGRFTISRVNAKNTVYLQMTSLKPEDTAVYYCNTGGVYSHPDYYTGTYWGQGTQVTVSS

SEQ ID NO: 32 - protein, 122 aa, Artificial Sequence
  Synthetic polypeptide
EVQVVESGGGLVQAGGSLRLSCAASGITFSSYAMGWYRQAPGKQRELVAAINRFGLTNYADSVKGRFTISRDNAKSTVYLQMTSLKPEDTAVYYCNTGGVYSHPDYYTGTYWGQGTQVTVSS

SEQ ID NO: 33 - protein, 122 aa, Artificial Sequence
  Synthetic polypeptide
EVQLVESGGGLVQAGGSLRLSCAASGITFSSYAMAWYRQDPGKQRELVAAINRFGLTNYADSVKGRFTISRDNAKNTVYLEMTSLKPEDTAVYYCNTGGVYSHPNYYTGTYWGQGTQVTVSS

SEQ ID NO: 34 - protein, 112 aa, Artificial Sequence
  Synthetic polypeptide
EVQLVESGGGLVQAGGSLRLSCVASTSTLTTYAVRWYRQAPGKQREWVAFISVDGNTNYPDSVKGRFIVSRDNAKNTVYLQMNSLKPEDTADYICRAGGQYWGQGTQVTVSS

SEQ ID NO: 35 - protein, 344 aa, Artificial Sequence
  Synthetic polypeptide
QVQLVESGGGLVQAGGSLRLSCVASRSTLTTYAVRWYRQAPGKQREWVAFISVDGNTNYPDSVKGRFIVSRDNAKNTVYLQMNSLKPEDTADYICRAGGQYWGQGTQVTVSSEPKSSDKTHTCPPCPAPEFEGGPSVFLFPPKPKDTLMISRTPEVTCVVVAVSHEDPEVKFNWYVDGVEVHNAKTKPREEQYNSTYRVVSVLTVLHQDWLNGKEYKCKVSNKALPAPIEKTISKAKGQPREPQVYTLPPSREEMTKNQVSLTCLVKGFYPSDIAVEWESNGQPENNYKTTPPVLDSDGSFFLYSKLTVDKSRWQQGNVFSCSVMHEALHNHYTQKSLSLSPGK

SEQ ID NO: 36 - protein, 354 aa, Artificial Sequence
  Synthetic polypeptide
EVQLVESGGGLVQAGGSLRLSCATSGITFSSYAMGWYRQAPGKQRELVAGINRFGLTNYADSVKGRFTISRDNAKNTVYLQMTSLKSEDTAVYYCNTGGVYSHPNYYTGIYWGQGTQVTVSSEPKSSDKTHTCPPCPAPEFEGGPSVFLFPPKPKDTLMISRTPEVTCVVVAVSHEDPEVKFNWYVDGVEVHNAKTKPREEQYNSTYRVVSVLTVLHQDWLNGKEYKCKVSNKALPAPIEKTISKAKGQPREPQVYTLPPSREEMTKNQVSLTCLVKGFYPSDIAVEWESNGQPENNYKTTPPVLDSDGSFFLYSKLTVDKSRWQQGNVFSCSVMHEALHNHYTQKSLSLSPGK

SEQ ID NO: 37 - protein, 344 aa, Artificial Sequence
  Synthetic polypeptide
QVQLVESGGGLVQAGGSLRLSCVGSSSTLTTYAVRWYRQAPGKQREWVAFISVDGNTNYPDSVKGRFIVSRDNAKNTVYLQMNNLKPEDTADYICRAGGQYWGQGTQVTVSSEPKSSDKTHTCPPCPAPEFEGGPSVFLFPPKPKDTLMISRTPEVTCVVVAVSHEDPEVKFNWYVDGVEVHNAKTKPREEQYNSTYRVVSVLTVLHQDWLNGKEYKCKVSNKALPAPIEKTISKAKGQPREPQVYTLPPSREEMTKNQVSLTCLVKGFYPSDIAVEWESNGQPENNYKTTPPVLDSDGSFFLYSKLTVDKSRWQQGNVFSCSVMHEALHNHYTQKSLSLSPGK

SEQ ID NO: 38 - protein, 344 aa, Artificial Sequence
  Synthetic polypeptide
QVQLVESGGGLVQAGGSLRLSCVASSSTVTTYAVRWYRQAPGKQREWVAFISVDGNTNYPDSVKGRFIVSRDNAKNTVYLQMNSLKPEDTADYICRAGGQYWGQGTQVTVSSEPKSSDKTHTCPPCPAPEFEGGPSVFLFPPKPKDTLMISRTPEVTCVVVAVSHEDPEVKFNWYVDGVEVHNAKTKPREEQYNSTYRVVSVLTVLHQDWLNGKEYKCKVSNKALPAPIEKTISKAKGQPREPQVYTLPPSREEMTKNQVSLTCLVKGFYPSDIAVEWESNGQPENNYKTTPPVLDSDGSFFLYSKLTVDKSRWQQGNVFSCSVMHEALHNHYTQKSLSLSPGK

SEQ ID NO: 39 - protein, 344 aa, Artificial Sequence
  Synthetic polypeptide
EVQLVESGGGLVQAGGSLRLSCVASGSTWTTYAVRWYRQAPGKQREWVAFISVDGSTNYPDSVKGRFIVSRDNAKNTVYLQMNSLKPEDTADYICRVGGQYWGQGTQVTVSSEPKSSDKTHTCPPCPAPEFEGGPSVFLFPPKPKDTLMISRTPEVTCVVVAVSHEDPEVKFNWYVDGVEVHNAKTKPREEQYNSTYRVVSVLTVLHQDWLNGKEYKCKVSNKALPAPIEKTISKAKGQPREPQVYTLPPSREEMTKNQVSLTCLVKGFYPSDIAVEWESNGQPENNYKTTPPVLDSDGSFFLYSKLTVDKSRWQQGNVFSCSVMHEALHNHYTQKSLSLSPGK

SEQ ID NO: 40 - protein, 344 aa, Artificial Sequence
  Synthetic polypeptide
EVQLVESGGGLVQAGGSLRLSCVASRSTLTTYAVRWYRQAPGKQREWVAFISVDGKTNYPDSVKGRFIVSRDNAKNTVYLQMNSLKPEDTADYICRAGGQYWGQGTQVTVSSEPKSSDKTHTCPPCPAPEFEGGPSVFLFPPKPKDTLMISRTPEVTCVVVAVSHEDPEVKFNWYVDGVEVHNAKTKPREEQYNSTYRVVSVLTVLHQDWLNGKEYKCKVSNKALPAPIEKTISKAKGQPREPQVYTLPPSREEMTKNQVSLTCLVKGFYPSDIAVEWESNGQPENNYKTTPPVLDSDGSFFLYSKLTVDKSRWQQGNVFSCSVMHEALHNHYTQKSLSLSPGK

SEQ ID NO: 41 - protein, 344 aa, Artificial Sequence
  Synthetic polypeptide
EVQVVESGGGLVQAGGSLRLSCVASRSTLSTYAVRWYRQAPGNQREWVAFISVDGNTNYPDSVKGRFIVSRDNAKNTVYLQMNSLKPEDTADYICRAGGQYWGQGTQVTVSSEPKSSDKTHTCPPCPAPEFEGGPSVFLFPPKPKDTLMISRTPEVTCVVVAVSHEDPEVKFNWYVDGVEVHNAKTKPREEQYNSTYRVVSVLTVLHQDWLNGKEYKCKVSNKALPAPIEKTISKAKGQPREPQVYTLPPSREEMTKNQVSLTCLVKGFYPSDIAVEWESNGQPENNYKTTPPVLDSDGSFFLYSKLTVDKSRWQQGNVFSCSVMHEALHNHYTQKSLSLSPGK

SEQ ID NO: 42 - protein, 344 aa, Artificial Sequence
  Synthetic polypeptide
EVQVVESGGGLVQAGGSLRLSCVASTSTLTTYAVRWYRQAPGKQREWVAFISVDGNTNYPDSVKGRFIVSRDNAKNTVYLQMNSLKPEDTADYICRAGGQYWGQGTQVTVSSEPKSSDKTHTCPPCPAPEFEGGPSVFLFPPKPKDTLMISRTPEVTCVVVAVSHEDPEVKFNWYVDGVEVHNAKTKPREEQYNSTYRVVSVLTVLHQDWLNGKEYKCKVSNKALPAPIEKTISKAKGQPREPQVYTLPPSREEMTKNQVSLTCLVKGFYPSDIAVEWESNGQPENNYKTTPPVLDSDGSFFLYSKLTVDKSRWQQGNVFSCSVMHEALHNHYTQKSLSLSPGK

SEQ ID NO: 43 - protein, 344 aa, Artificial Sequence
  Synthetic polypeptide
QVQLVESGGGLVQAGGSLRLSCVGSSSTLTTYAVRWYRQAPGKQREWVAFISVDGSTNYPDSVKGRFIVSRDNAKNTVYLQMNSLKPEDTADYICRAGGQYWGQGTQVTVSSEPKSSDKTHTCPPCPAPEFEGGPSVFLFPPKPKDTLMISRTPEVTCVVVAVSHEDPEVKFNWYVDGVEVHNAKTKPREEQYNSTYRVVSVLTVLHQDWLNGKEYKCKVSNKALPAPIEKTISKAKGQPREPQVYTLPPSREEMTKNQVSLTCLVKGFYPSDIAVEWESNGQPENNYKTTPPVLDSDGSFFLYSKLTVDKSRWQQGNVFSCSVMHEALHNHYTQKSLSLSPGK

SEQ ID NO: 44 - protein, 354 aa, Artificial Sequence
  Synthetic polypeptide
EVQVVESGGGLAQAGGSLRLSCAVSGITFSSYAMGWYRQDPGKQRELVAAINRFGLTNYADSVKGRFTISRDNAKNTVYLQMTSLKPEDTAVYYCNTGGVYSHPNYYTGTYWGQGTQVTVSSEPKSSDKTHTCPPCPAPEFEGGPSVFLFPPKPKDTLMISRTPEVTCVVVAVSHEDPEVKFNWYVDGVEVHNAKTKPREEQYNSTYRVVSVLTVLHQDWLNGKEYKCKVSNKALPAPIEKTISKAKGQPREPQVYTLPPSREEMTKNQVSLTCLVKGFYPSDIAVEWESNGQPENNYKTTPPVLDSDGSFFLYSKLTVDKSRWQQGNVFSCSVMHEALHNHYTQKSLSLSPGK

SEQ ID NO: 45 - protein, 354 aa, Artificial Sequence
  Synthetic polypeptide
QVQLVESGGGLVQAGGSLRLSCAASGITFSSYAMGWYRQAPGKQRELVAAINRFGLTNYADFVKGRFTISRVNAKNTVYLQMTSLKPEDTAVYYCNTGGVYSHPDYYTGTYWGQGTQVTVSSEPKSSDKTHTCPPCPAPEFEGGPSVFLFPPKPKDTLMISRTPEVTCVVVAVSHEDPEVKFNWYVDGVEVHNAKTKPREEQYNSTYRVVSVLTVLHQDWLNGKEYKCKVSNKALPAPIEKTISKAKGQPREPQVYTLPPSREEMTKNQVSLTCLVKGFYPSDIAVEWESNGQPENNYKTTPPVLDSDGSFFLYSKLTVDKSRWQQGNVFSCSVMHEALHNHYTQKSLSLSPGK

SEQ ID NO: 46 - protein, 354 aa, Artificial Sequence
  Synthetic polypeptide
EVQVVESGGGLVQAGGSLRLSCAASGITFSSYAMGWYRQAPGKQRELVAAINRFGLTNYADSVKGRFTISRDNAKSTVYLQMTSLKPEDTAVYYCNTGGVYSHPDYYTGTYWGQGTQVTVSSEPKSSDKTHTCPPCPAPEFEGGPSVFLFPPKPKDTLMISRTPEVTCVVVAVSHEDPEVKFNWYVDGVEVHNAKTKPREEQYNSTYRVVSVLTVLHQDWLNGKEYKCKVSNKALPAPIEKTISKAKGQPREPQVYTLPPSREEMTKNQVSLTCLVKGFYPSDIAVEWESNGQPENNYKTTPPVLDSDGSFFLYSKLTVDKSRWQQGNVFSCSVMHEALHNHYTQKSLSLSPGK

SEQ ID NO: 47 - protein, 354 aa, Artificial Sequence
  Synthetic polypeptide
EVQLVESGGGLVQAGGSLRLSCAASGITFSSYAMAWYRQDPGKQRELVAAINRFGLTNYADSVKGRFTISRDNAKNTVYLEMTSLKPEDTAVYYCNTGGVYSHPNYYTGTYWGQGTQVTVSSEPKSSDKTHTCPPCPAPEFEGGPSVFLFPPKPKDTLMISRTPEVTCVVVAVSHEDPEVKFNWYVDGVEVHNAKTKPREEQYNSTYRVVSVLTVLHQDWLNGKEYKCKVSNKALPAPIEKTISKAKGQPREPQVYTLPPSREEMTKNQVSLTCLVKGFYPSDIAVEWESNGQPENNYKTTPPVLDSDGSFFLYSKLTVDKSRWQQGNVFSCSVMHEALHNHYTQKSLSLSPGK

SEQ ID NO: 48 - protein, 344 aa, Artificial Sequence
  Synthetic polypeptide
EVQLVESGGGLVQAGGSLRLSCVASTSTLTTYAVRWYRQAPGKQREWVAFISVDGNTNYPDSVKGRFIVSRDNAKNTVYLQMNSLKPEDTADYICRAGGQYWGQGTQVTVSSEPKSSDKTHTCPPCPAPEFEGGPSVFLFPPKPKDTLMISRTPEVTCVVVAVSHEDPEVKFNWYVDGVEVHNAKTKPREEQYNSTYRVVSVLTVLHQDWLNGKEYKCKVSNKALPAPIEKTISKAKGQPREPQVYTLPPSREEMTKNQVSLTCLVKGFYPSDIAVEWESNGQPENNYKTTPPVLDSDGSFFLYSKLTVDKSRWQQGNVFSCSVMHEALHNHYTQKSLSLSPGK

SEQ ID NO: 49 - protein, 5 aa, Artificial Sequence
  Synthetic polypeptide
TYAVR

SEQ ID NO: 50 - protein, 16 aa, Artificial Sequence
  Synthetic polypeptide
FISVDGNTNYPDSVKG

SEQ ID NO: 51 - protein, 4 aa, Artificial Sequence
  Synthetic polypeptide
GGQY

SEQ ID NO: 52 - protein, 7 aa, Artificial Sequence
  Synthetic polypeptide
RSTLTTY

SEQ ID NO: 53 - protein, 5 aa, Artificial Sequence
  Synthetic polypeptide
SVDGN

SEQ ID NO: 54 - protein, 8 aa, Artificial Sequence
  Synthetic polypeptide
RSTLTTYA

SEQ ID NO: 55 - protein, 7 aa, Artificial Sequence
  Synthetic polypeptide
ISVDGNT

SEQ ID NO: 56 - protein, 6 aa, Artificial Sequence
  Synthetic polypeptide
RAGGQY

SEQ ID NO: 57 - protein, 5 aa, Artificial Sequence
  Synthetic polypeptide
SYAMG

SEQ ID NO: 58 - protein, 16 aa, Artificial Sequence
  Synthetic polypeptide
GINRFGLTNYADSVKG

SEQ ID NO: 59 - protein, 14 aa, Artificial Sequence
  Synthetic polypeptide
GGVYSHPNYYTGIY

SEQ ID NO: 60 - protein, 7 aa, Artificial Sequence
  Synthetic polypeptide
GITFSSY

SEQ ID NO: 61 - protein, 5 aa, Artificial Sequence
  Synthetic polypeptide
NRFGL

SEQ ID NO: 62 - protein, 8 aa, Artificial Sequence
  Synthetic polypeptide
GITFSSYA

SEQ ID NO: 63 - protein, 7 aa, Artificial Sequence
  Synthetic polypeptide
INRFGLT

SEQ ID NO: 64 - protein, 16 aa, Artificial Sequence
  Synthetic polypeptide
NTGGVYSHPNYYTGIY

SEQ ID NO: 65 - protein, 7 aa, Artificial Sequence
  Synthetic polypeptide
SSTLTTY

SEQ ID NO: 66 - protein, 8 aa, Artificial Sequence
  Synthetic polypeptide
SSTLTTYA

SEQ ID NO: 67 - protein, 7 aa, Artificial Sequence
  Synthetic polypeptide
SSTVTTY

SEQ ID NO: 68 - protein, 8 aa, Artificial Sequence
  Synthetic polypeptide
SSTVTTYA

SEQ ID NO: 69 - protein, 16 aa, Artificial Sequence
  Synthetic polypeptide
FISVDGSTNYPDSVKG

SEQ ID NO: 70 - protein, 7 aa, Artificial Sequence
  Synthetic polypeptide
GSTWTTY

SEQ ID NO: 71 - protein, 5 aa, Artificial Sequence
  Synthetic polypeptide
SVDGS

SEQ ID NO: 72 - protein, 8 aa, Artificial Sequence
  Synthetic polypeptide
GSTWTTYA

SEQ ID NO: 73 - protein, 7 aa, Artificial Sequence
  Synthetic polypeptide
ISVDGST

SEQ ID NO: 74 - protein, 6 aa, Artificial Sequence
  Synthetic polypeptide
RVGGQY

SEQ ID NO: 75 - protein, 16 aa, Artificial Sequence
  Synthetic polypeptide
FISVDGKTNYPDSVKG

SEQ ID NO: 76 - protein, 5 aa, Artificial Sequence
  Synthetic polypeptide
SVDGK

SEQ ID NO: 77 - protein, 7 aa, Artificial Sequence
  Synthetic polypeptide
ISVDGKT

SEQ ID NO: 78 - protein, 7 aa, Artificial Sequence
  Synthetic polypeptide
RSTLSTY

SEQ ID NO: 79 - protein, 8 aa, Artificial Sequence
  Synthetic polypeptide
RSTLSTYA

SEQ ID NO: 80 - protein, 7 aa, Artificial Sequence
  Synthetic polypeptide
TSTLTTY

SEQ ID NO: 81 - protein, 8 aa, Artificial Sequence
  Synthetic polypeptide
TSTLTTYA

SEQ ID NO: 82 - protein, 16 aa, Artificial Sequence
  Synthetic polypeptide
AINRFGLTNYADSVKG

SEQ ID NO: 83 - protein, 14 aa, Artificial Sequence
  Synthetic polypeptide
GGVYSHPNYYTGTY

SEQ ID NO: 84 - protein, 16 aa, Artificial Sequence
  Synthetic polypeptide
NTGGVYSHPNYYTGTY

SEQ ID NO: 85 - protein, 16 aa, Artificial Sequence
  Synthetic polypeptide
AINRFGLTNYADFVKG

SEQ ID NO: 86 - protein, 14 aa, Artificial Sequence
  Synthetic polypeptide
GGVYSHPDYYTGTY

SEQ ID NO: 87 - protein, 16 aa, Artificial Sequence
  Synthetic polypeptide
NTGGVYSHPDYYTGTY

SEQ ID NO: 88 - protein, 5 aa, Artificial Sequence
  Synthetic polypeptide
SYAMA

SEQ ID NO: 89 - protein, 232 aa, Artificial Sequence
  Synthetic polypeptide
EPKSSDKTHTCPPCPAPEFEGGPSVFLFPPKPKDTLMISRTPEVTCVVVAVSHEDPEVKFNWYVDGVEVHNAKTKPREEQYNSTYRVVSVLTVLHQDWLNGKEYKCKVSNKALPAPIEKTISKAKGQPREPQVYTLPPSREEMTKNQVSLTCLVKGFYPSDIAVEWESNGQPENNYKTTPPVLDSDGSFFLYSKLTVDKSRWQQGNVFSCSVMHEALHNHYTQKSLSLSPGK

SEQ ID NO: 90 - protein, 112 aa, Artificial Sequence
  Synthetic polypeptide
EVQLVESGGGVVQPGGSLRLSCAASGSTWTTYAVRWYRQAPGKQREWVAFISVDGSTNYADSVKGRFTISRDNSKNTVYLQMNSLRAEDTADYICRVGGQYWGQGTMVTVSS

SEQ ID NO: 91 - protein, 112 aa, Artificial Sequence
  Synthetic polypeptide
EVQLVESGGGVVQPGGSLRLSCAASGSTWTTYAVRWYRQAPGKQREWVAFISVDGSTNYPDSVKGRFTISRDNSKNTVYLQMNSLRAEDTADYICRVGGQYWGQGTMVTVSS

SEQ ID NO: 92 - protein, 112 aa, Artificial Sequence
  Synthetic polypeptide
EVQLVESGGGVVQPGGSLRLSCAASGSTWTTYAVRWYRQAPGKQREWVAFISVDGSTNYADSVKGRFTISRDNAKNTVYLQMNSLRAEDTADYICRVGGQYWGQGTMVTVSS

SEQ ID NO: 93 - protein, 112 aa, Artificial Sequence
  Synthetic polypeptide
EVQLVESGGGVVQPGGSLRLSCAASGSTWTTYAVRWYRQAPGKQREWVAFISVDGSTNYADSVKGRFTVSRDNSKNTVYLQMNSLRAEDTADYICRVGGQYWGQGTMVTVSS

SEQ ID NO: 94 - protein, 112 aa, Artificial Sequence
  Synthetic polypeptide
EVQLVESGGGVVQPGGSLRLSCAASGSTWTTYAVRWYRQAPGKQREWVAFISVDGSTNYADSVKGRFTISRDNSKNTVYLQMNSLRAEDTADYICRVGGQYWGQGTQVTVSS

SEQ ID NO: 95 - protein, 122 aa, Artificial Sequence
  Synthetic polypeptide
EVQLVESGGGLVQPGGSLRLSCAASGITFSSYAMGWYRQAPGKQRELVAAINRFGLTYYVDSVKGRFTISRDNAKNSLYLQMNSLRAEDTAVYYCNTGGVYSHPDYYTGTYWGQGTMVTVSS

SEQ ID NO: 96 - protein, 122 aa, Artificial Sequence
  Synthetic polypeptide
EVQLVESGGGLVQPGGSLRLSCAASGITFSSYAMGWYRQAPGKQRELVAAINRFGLTNYVDSVKGRFTISRDNAKNSLYLQMNSLRAEDTAVYYCNTGGVYSHPDYYTGTYWGQGTMVTVSS

SEQ ID NO: 97 - protein, 122 aa, Artificial Sequence
  Synthetic polypeptide
EVQLVESGGGLVQPGGSLRLSCAASGITFSSYAMGWYRQAPGKQRELVAAINRFGLTNYADFVKGRFTISRDNAKNSLYLQMNSLRAEDTAVYYCNTGGVYSHPDYYTGTYWGQGTMVTVSS

SEQ ID NO: 98 - protein, 122 aa, Artificial Sequence
  Synthetic polypeptide
EVQLVESGGGLVQPGGSLRLSCAASGITFSSYAMGWYRQAPGKQRELVAAINRFGLTNYVDSVKGRFTISRVNAKNSLYLQMNSLRAEDTAVYYCNTGGVYSHPDYYTGTYWGQGTMVTVSS

SEQ ID NO: 99 - protein, 122 aa, Artificial Sequence
  Synthetic polypeptide
EVQLVESGGGLVQPGGSLRLSCAASGITFSSYAMGWYRQAPGKQRELVAAINRFGLTNYVDSVKGRFTISRDNAKNSVYLQMNSLRAEDTAVYYCNTGGVYSHPDYYTGTYWGQGTMVTVSS

SEQ ID NO: 100 - protein, 122 aa, Artificial Sequence
  Synthetic polypeptide
EVQLVESGGGLVQPGGSLRLSCAASGITFSSYAMGWYRQAPGKQRELVAAINRFGLTNYVDSVKGRFTISRDNAKNSLYLQMNSLRAEDTAVYYCNTGGVYSHPDYYTGTYWGQGTQVTVSS

SEQ ID NO: 101 - protein, 122 aa, Artificial Sequence
  Synthetic polypeptide
EVQLVESGGGLVQPGGSLRLSCAASGITFSSYAMGWYRQAPGKQRELVAAINRFGLTNYADFVKGRFTISRVNAKNSLYLQMNSLRAEDTAVYYCNTGGVYSHPDYYTGTYWGQGTMVTVSS

SEQ ID NO: 102 - protein, 344 aa, Artificial Sequence
  Synthetic polypeptide
EVQLVESGGGVVQPGGSLRLSCAASGSTWTTYAVRWYRQAPGKQREWVAFISVDGSTNYADSVKGRFTISRDNSKNTVYLQMNSLRAEDTADYICRVGGQYWGQGTMVTVSSEPKSSDKTHTCPPCPAPEEFGGPSVFLFPPKPKDTLMISRTPEVTCVVVAVSHEDPEVKFNWYVDGVEVHNAKTKPREEQYNSTYRVVSVLTVLHQDWLNGKEYKCKVSNKALPAPIEKTISKAKGQPREPQVYTLPPSREEMTKNQVSLTCLVKGFYPSDIAVEWESNGQPENNYKTTPPVLDSDGSFFLYSKLTVDKSRWQQGNVFSCSVMHEALHNHYTQKSLSLSPGK

SEQ ID NO: 103 - protein, 344 aa, Artificial Sequence
  Synthetic polypeptide
EVQLVESGGGVVQPGGSLRLSCAASGSTWTTYAVRWYRQAPGKQREWVAFISVDGSTNYPDSVKGRFTISRDNSKNTVYLQMNSLRAEDTADYICRVGGQYWGQGTMVTVSSEPKSSDKTHTCPPCPAPEEFGGPSVFLFPPKPKDTLMISRTPEVTCVVVAVSHEDPEVKFNWYVDGVEVHNAKTKPREEQYNSTYRVVSVLTVLHQDWLNGKEYKCKVSNKALPAPIEKTISKAKGQPREPQVYTLPPSREEMTKNQVSLTCLVKGFYPSDIAVEWESNGQPENNYKTTPPVLDSDGSFFLYSKLTVDKSRWQQGNVFSCSVMHEALHNHYTQKSLSLSPGK

SEQ ID NO: 104 - protein, 344 aa, Artificial Sequence
  Synthetic polypeptide
EVQLVESGGGVVQPGGSLRLSCAASGSTWTTYAVRWYRQAPGKQREWVAFISVDGSTNYADSVKGRFTISRDNAKNTVYLQMNSLRAEDTADYICRVGGQYWGQGTMVTVSSEPKSSDKTHTCPPCPAPEEFGGPSVFLFPPKPKDTLMISRTPEVTCVVVAVSHEDPEVKFNWYVDGVEVHNAKTKPREEQYNSTYRVVSVLTVLHQDWLNGKEYKCKVSNKALPAPIEKTISKAKGQPREPQVYTLPPSREEMTKNQVSLTCLVKGFYPSDIAVEWESNGQPENNYKTTPPVLDSDGSFFLYSKLTVDKSRWQQGNVFSCSVMHEALHNHYTQKSLSLSPGK

SEQ ID NO: 105 - protein, 344 aa, Artificial Sequence
  Synthetic polypeptide
EVQLVESGGGVVQPGGSLRLSCAASGSTWTTYAVRWYRQAPGKQREWVAFISVDGSTNYADSVKGRFTVSRDNSKNTVYLQMNSLRAEDTADYICRVGGQYWGQGTMVTVSSEPKSSDKTHTCPPCPAPEEFGGPSVFLFPPKPKDTLMISRTPEVTCVVVAVSHEDPEVKFNWYVDGVEVHNAKTKPREEQYNSTYRVVSVLTVLHQDWLNGKEYKCKVSNKALPAPIEKTISKAKGQPREPQVYTLPPSREEMTKNQVSLTCLVKGFYPSDIAVEWESNGQPENNYKTTPPVLDSDGSFFLYSKLTVDKSRWQQGNVFSCSVMHEALHNHYTQKSLSLSPGK

SEQ ID NO: 106 - protein, 344 aa, Artificial Sequence
  Synthetic polypeptide
EVQLVESGGGVVQPGGSLRLSCAASGSTWTTYAVRWYRQAPGKQREWVAFISVDGSTNYADSVKGRFTISRDNSKNTVYLQMNSLRAEDTADYICRVGGQYWGQGTQVTVSSEPKSSDKTHTCPPCPAPEEFGGPSVFLFPPKPKDTLMISRTPEVTCVVVAVSHEDPEVKFNWYVDGVEVHNAKTKPREEQYNSTYRVVSVLTVLHQDWLNGKEYKCKVSNKALPAPIEKTISKAKGQPREPQVYTLPPSREEMTKNQVSLTCLVKGFYPSDIAVEWESNGQPENNYKTTPPVLDSDGSFFLYSKLTVDKSRWQQGNVFSCSVMHEALHNHYTQKSLSLSPGK

SEQ ID NO: 107 - protein, 354 aa, Artificial Sequence
  Synthetic polypeptide
EVQLVESGGGLVQPGGSLRLSCAASGITFSSYAMGWYRQAPGKQRELVAAINRFGLTYYVDSVKGRFTISRDNAKNSLYLQMNSLRAEDTAVYYCNTGGVYSHPDYYTGTYWGQGTMVTVSSEPKSSDKTHTCPPCPAPEEFGGPSVFLFPPKPKDTLMISRTPEVTCVVVAVSHEDPEVKFNWYVDGVEVHNAKTKPREEQYNSTYRVVSVLTVLHQDWLNGKEYKCKVSNKALPAPIEKTISKAKGQPREPQVYTLPPSREEMTKNQVSLTCLVKGFYPSDIAVEWESNGQPENNYKTTPPVLDSDGSFFLYSKLTVDKSRWQQGNVFSCSVMHEALHNHYTQKSLSLSPGK

SEQ ID NO: 108 - protein, 354 aa, Artificial Sequence
  Synthetic polypeptide
EVQLVESGGGLVQPGGSLRLSCAASGITFSSYAMGWYRQAPGKQRELVAAINRFGLTNYVDSVKGRFTISRDNAKNSLYLQMNSLRAEDTAVYYCNTGGVYSHPDYYTGTYWGQGTMVTVSSEPKSSDKTHTCPPCPAPEEFGGPSVFLFPPKPKDTLMISRTPEVTCVVVAVSHEDPEVKFNWYVDGVEVHNAKTKPREEQYNSTYRVVSVLTVLHQDWLNGKEYKCKVSNKALPAPIEKTISKAKGQPREPQVYTLPPSREEMTKNQVSLTCLVKGFYPSDIAVEWESNGQPENNYKTTPPVLDSDGSFFLYSKLTVDKSRWQQGNVFSCSVMHEALHNHYTQKSLSLSPGK

SEQ ID NO: 109 - protein, 354 aa, Artificial Sequence
  Synthetic polypeptide
EVQLVESGGGLVQPGGSLRLSCAASGITFSSYAMGWYRQAPGKQRELVAAINRFGLTNYADFVKGRFTISRDNAKNSLYLQMNSLRAEDTAVYYCNTGGVYSHPDYYTGTYWGQGTMVTVSSEPKSSDKTHTCPPCPAPEEFGGPSVFLFPPKPKDTLMISRTPEVTCVVVAVSHEDPEVKFNWYVDGVEVHNAKTKPREEQYNSTYRVVSVLTVLHQDWLNGKEYKCKVSNKALPAPIEKTISKAKGQPREPQVYTLPPSREEMTKNQVSLTCLVKGFYPSDIAVEWESNGQPENNYKTTPPVLDSDGSFFLYSKLTVDKSRWQQGNVFSCSVMHEALHNHYTQKSLSLSPGK

SEQ ID NO: 110 - protein, 354 aa, Artificial Sequence
  Synthetic polypeptide
EVQLVESGGGLVQPGGSLRLSCAASGITFSSYAMGWYRQAPGKQRELVAAINRFGLTNYVDSVKGRFTISRVNAKNSLYLQMNSLRAEDTAVYYCNTGGVYSHPDYYTGTYWGQGTMVTVSSEPKSSDKTHTCPPCPAPEEFGGPSVFLFPPKPKDTLMISRTPEVTCVVVAVSHEDPEVKFNWYVDGVEVHNAKTKPREEQYNSTYRVVSVLTVLHQDWLNGKEYKCKVSNKALPAPIEKTISKAKGQPREPQVYTLPPSREEMTKNQVSLTCLVKGFYPSDIAVEWESNGQPENNYKTTPPVLDSDGSFFLYSKLTVDKSRWQQGNVFSCSVMHEALHNHYTQKSLSLSPGK

SEQ ID NO: 111 - protein, 354 aa, Artificial Sequence
  Synthetic polypeptide
EVQLVESGGGLVQPGGSLRLSCAASGITFSSYAMGWYRQAPGKQRELVAAINRFGLTNYVDSVKGRFTISRDNAKNSVYLQMNSLRAEDTAVYYCNTGGVYSHPDYYTGTYWGQGTMVTVSSEPKSSDKTHTCPPCPAPEEFGGPSVFLFPPKPKDTLMISRTPEVTCVVVAVSHEDPEVKFNWYVDGVEVHNAKTKPREEQYNSTYRVVSVLTVLHQDWLNGKEYKCKVSNKALPAPIEKTISKAKGQPREPQVYTLPPSREEMTKNQVSLTCLVKGFYPSDIAVEWESNGQPENNYKTTPPVLDSDGSFFLYSKLTVDKSRWQQGNVFSCSVMHEALHNHYTQKSLSLSPGK

SEQ ID NO: 112 - protein, 354 aa, Artificial Sequence
  Synthetic polypeptide
EVQLVESGGGLVQPGGSLRLSCAASGITFSSYAMGWYRQAPGKQRELVAAINRFGLTNYVDSVKGRFTISRDNAKNSLYLQMNSLRAEDTAVYYCNTGGVYSHPDYYTGTYWGQGTQVTVSSEPKSSDKTHTCPPCPAPEEFGGPSVFLFPPKPKDTLMISRTPEVTCVVVAVSHEDPEVKFNWYVDGVEVHNAKTKPREEQYNSTYRVVSVLTVLHQDWLNGKEYKCKVSNKALPAPIEKTISKAKGQPREPQVYTLPPSREEMTKNQVSLTCLVKGFYPSDIAVEWESNGQPENNYKTTPPVLDSDGSFFLYSKLTVDKSRWQQGNVFSCSVMHEALHNHYTQKSLSLSPGK

SEQ ID NO: 113 - protein, 354 aa, Artificial Sequence
  Synthetic polypeptide
EVQLVESGGGLVQPGGSLRLSCAASGITFSSYAMGWYRQAPGKQRELVAAINRFGLTNYADFVKGRFTISRVNAKNSLYLQMNSLRAEDTAVYYCNTGGVYSHPDYYTGTYWGQGTMVTVSSEPKSSDKTHTCPPCPAPEEFGGPSVFLFPPKPKDTLMISRTPEVTCVVVAVSHEDPEVKFNWYVDGVEVHNAKTKPREEQYNSTYRVVSVLTVLHQDWLNGKEYKCKVSNKALPAPIEKTISKAKGQPREPQVYTLPPSREEMTKNQVSLTCLVKGFYPSDIAVEWESNGQPENNYKTTPPVLDSDGSFFLYSKLTVDKSRWQQGNVFSCSVMHEALHNHYTQKSLSLSPGK